European Patent Application EP 4 269 580 A1, published November 1, 2023. Title: Method of inducing large deletion in genomic DNA and method of analyzing the deletion. Applicant: Logomix, Inc. The sequence listing filed with the application follows.

SEQUENCE LISTING (388 sequences)

SEQ ID NO: 1 - DNA, 25 bp, Artificial Sequence
  L1 forward primer
caccgaataattgtgtagttaagtc

SEQ ID NO: 2 - DNA, 25 bp, Artificial Sequence
  L1 reverse primer
aaacgacttaactacacaattattc

SEQ ID NO: 3 - DNA, 25 bp, Artificial Sequence
  L2 forward primer
caccgttaatagcttgatatagcta

SEQ ID NO: 4 - DNA, 25 bp, Artificial Sequence
  L2 reverse primer
aaactagctatatcaagctattaac

SEQ ID NO: 5 - DNA, 25 bp, Artificial Sequence
  L3 formard primer
caccggggagagattatgctttacg

SEQ ID NO: 6 - DNA, 25 bp, Artificial Sequence
  L3 reverse primer
aaaccgtaaagcataatctctcccc

SEQ ID NO: 7 - DNA, 25 bp, Artificial Sequence
  L4 forward primer
caccgttctcagcaattgtgcggtc

SEQ ID NO: 8 - DNA, 25 bp, Artificial Sequence
  L4 reverse primer
aaacgaccgcacaattgctgagaac

SEQ ID NO: 9 - DNA, 25 bp, Artificial Sequence
  L5 forward primer
caccgcatctagcactcccggtaac

SEQ ID NO: 10 - DNA, 25 bp, Artificial Sequence
  L5 reverse primer
aaacgttaccgggagtgctagatgc

SEQ ID NO: 11 - DNA, 25 bp, Artificial Sequence
  L6 forward primer
caccgttctcagcaattgtgcggtc

SEQ ID NO: 12 - DNA, 25 bp, Artificial Sequence
  L6 reverse primer
aaacgaccgcacaattgctgagaac

SEQ ID NO: 13 - DNA, 25 bp, Artificial Sequence
  L7 forward primer
caccgtggggaagagctcaccgctc

SEQ ID NO: 14 - DNA, 25 bp, Artificial Sequence
  L7 reverse primer
aaacgagcggtgagctcttccccac

SEQ ID NO: 15 - DNA, 25 bp, Artificial Sequence
  L8 forward primer
caccgatccccattactagctcgaa

SEQ ID NO: 16 - DNA, 25 bp, Artificial Sequence
  L8 reverse primer
aaacttcgagctagtaatggggatc

SEQ ID NO: 17 - DNA, 25 bp, Artificial Sequence
  L9 forward primer
caccgatttctatgaacacacgtag

SEQ ID NO: 18 - DNA, 25 bp, Artificial Sequence
  L9 reverse primer
aaacctacgtgtgttcatagaaatc

SEQ ID NO: 19 - DNA, 25 bp, Artificial Sequence
  L10 forward primer
caccggcatggagtgaatacgactt

SEQ ID NO: 20 - DNA, 25 bp, Artificial Sequence
  L10 reverse primer
aaacaagtcgtattcactccatgcc

SEQ ID NO: 21 - DNA, 25 bp, Artificial Sequence
  L11 forward primer
caccgcagagaaatgacgaacgatt

SEQ ID NO: 22 - DNA, 25 bp, Artificial Sequence
  L11 reverser primer
aaacaatcgttcgtcatttctctgc

SEQ ID NO: 23 - DNA, 25 bp, Artificial Sequence
  L12 forward primer
caccgagcacatttgcaacgtcacg

SEQ ID NO: 24 - DNA, 25 bp, Artificial Sequence
  L12 reverse primer
aaaccgtgacgttgcaaatgtgctc

SEQ ID NO: 25 - DNA, 25 bp, Artificial Sequence
  R1 forward primer
caccggacagcagtgagcgtagagt

SEQ ID NO: 26 - DNA, 25 bp, Artificial Sequence
  R1 reverse primer
aaacactctacgctcactgctgtcc

SEQ ID NO: 27 - DNA, 25 bp, Artificial Sequence
  R2 forward primer
caccgcacttgatgcattaatgccg

SEQ ID NO: 28 - DNA, 25 bp, Artificial Sequence
  R2 reverse primer
aaaccggcattaatgcatcaagtgc

SEQ ID NO: 29 - DNA, 25 bp, Artificial Sequence
  R3 forward primer
caccggagggagaaacaggtccgtt

SEQ ID NO: 30 - DNA, 25 bp, Artificial Sequence
  R3 reverse primer
aaacaacggacctgtttctccctcc

SEQ ID NO: 31 - DNA, 25 bp, Artificial Sequence
  R4 forward primer
caccgaacagaaaagtttactgcga

SEQ ID NO: 32 - DNA, 25 bp, Artificial Sequence
  R4 reverse primer
aaactcgcagtaaacttttctgttc

SEQ ID NO: 33 - DNA, 25 bp, Artificial Sequence
  R5 forward primer
caccgttactagaaaatgtgaaacg

SEQ ID NO: 34 - DNA, 25 bp, Artificial Sequence
  R5 reverse primer
aaaccgtttcacattttctagtaac

SEQ ID NO: 35 - DNA, 25 bp, Artificial Sequence
  R6 forward primer
caccgagaacagtgtgccagatcga

SEQ ID NO: 36 - DNA, 25 bp, Artificial Sequence
  R6 reverse primer
aaactcgatctggcacactgttctc

SEQ ID NO: 37 - DNA, 25 bp, Artificial Sequence
  R7 forward primer
caccgaagccaactacaactacgga

SEQ ID NO: 38 - DNA, 25 bp, Artificial Sequence
  R7 reverse primer
aaactccgtagttgtagttggcttc

SEQ ID NO: 39 - DNA, 25 bp, Artificial Sequence
  R8 forward primer
caccggctgtgctattaagatgcgc

SEQ ID NO: 40 - DNA, 25 bp, Artificial Sequence
  R8 reverse primer
aaacgcgcatcttaatagcacagcc

SEQ ID NO: 41 - DNA, 25 bp, Artificial Sequence
  R9 forward primer
caccgccatggactggaatagccgg

SEQ ID NO: 42 - DNA, 25 bp, Artificial Sequence
  R9 reverse primer
aaacccggctattccagtccatggc

SEQ ID NO: 43 - DNA, 25 bp, Artificial Sequence
  gRNA#1 forward primer
caccgagccccagcaagagcacaag

SEQ ID NO: 44 - DNA, 25 bp, Artificial Sequence
  gRNA#1 reverse primer
aaaccttgtgctcttgctggggctc

SEQ ID NO: 45 - DNA, 25 bp, Artificial Sequence
  gRNA#2 forward primer
caccggagatcgagtgccgcatcac

SEQ ID NO: 46 - DNA, 25 bp, Artificial Sequence
  gRNA#2 reverse primer
aaacgtgatgcggcactcgatctcc

SEQ ID NO: 47 - DNA, 25 bp, Artificial Sequence
  gRNA#3 forward primer
caccggggactgcagtcaagtcgaa

SEQ ID NO: 48 - DNA, 25 bp, Artificial Sequence
  gRNA#3 reverse primer
aaacttcgacttgactgcagtcccc

SEQ ID NO: 49 - DNA, 40 bp, Artificial Sequence
  HY1674
atatggccacaaccgccaccatgggtaccgtgagcaaggg

SEQ ID NO: 50 - DNA, 41 bp, Artificial Sequence
  HY1675
gacgactgagcgcgggatctcttgtacagctcgtccatgcc

SEQ ID NO: 51 - DNA, 40 bp, Artificial Sequence
  JS214
gatcgagtgccgcatcaccggcaattgacgcgtgctcctc

SEQ ID NO: 52 - DNA, 20 bp, Artificial Sequence
  HY1673
ggtggcggttgtggccatat

SEQ ID NO: 53 - DNA, 40 bp, Artificial Sequence
  JS210
aaactcatcaatgtatcttaattgcgttgcgctcactgcc

SEQ ID NO: 54 - DNA, 40 bp, Artificial Sequence
  JS211
gtgatgcggcactcgatctccctgatgcggtattttctcc

SEQ ID NO: 55 - DNA, 84 bp, Artificial Sequence
  HY2669
ccgcgctcagtcgtccaattctgccgtggacggcaccgccggacccggctccaccggatctcgcgagggcagaggaagtcttct

SEQ ID NO: 56 - DNA, 28 bp, Artificial Sequence
  JS218
taagatacattgatgagtttggacaaac

SEQ ID NO: 57 - DNA, 39 bp, Artificial Sequence
  HY1498
gaatactcattttagcttccttagctcctgaaaatctcg

SEQ ID NO: 58 - DNA, 39 bp, Artificial Sequence
  HY1499
gcatcgcaaactgcacccggtgccgggcagccacatcca

SEQ ID NO: 59 - DNA, 40 bp, Artificial Sequence
  HY1496
gcccgggcgcatgcgggccggatcagactatcagcgtgag

SEQ ID NO: 60 - DNA, 33 bp, Artificial Sequence
  HY1497
ggaagctaaaatgagtattcaacatttccgtgt

SEQ ID NO: 61 - DNA, 45 bp, Artificial Sequence
  HY1569
gtgggatccagacttcgaattcatgtcgaaagctacatataagga

SEQ ID NO: 62 - DNA, 49 bp, Artificial Sequence
  HY1570
tccggcccgcatgcgcccgggccggccctgatgcggtattttctcctta

SEQ ID NO: 63 - DNA, 44 bp, Artificial Sequence
  HY1567
aactcatcaatgtatcttagcccctacaacaactaagaaaatgg

SEQ ID NO: 64 - DNA, 45 bp, Artificial Sequence
  HY1568
gacatgaattcgaagtctggatcccactatttataccatgggagg

SEQ ID NO: 65 - DNA, 36 bp, Artificial Sequence
  HY2670
atatggccacaaccgccaccatgaccgagtacaagc

SEQ ID NO: 66 - DNA, 27 bp, Artificial Sequence
  HY1419
gctaagatacattgatgagtttggaca

SEQ ID NO: 67 - DNA, 40 bp, Artificial Sequence
  JS213
gtggcggttgtggccatattatcatcgtgtttttcaaagg

SEQ ID NO: 68 - DNA, 22 bp, Artificial Sequence
  HY1571
atcgtctttccctcgctatcac

SEQ ID NO: 69 - DNA, 24 bp, Artificial Sequence
  HY1572
ccactatttataccatgggaggcg

SEQ ID NO: 70 - DNA, 44 bp, Artificial Sequence
  HY1587
tcccatggtataaatagtggggcttataaatgcagatcctttac

SEQ ID NO: 71 - DNA, 21 bp, Artificial Sequence
  HY1578
ctgccaagaaggagaacagag

SEQ ID NO: 72 - DNA, 22 bp, Artificial Sequence
  HY1579
aatacctctgctgaacctacca

SEQ ID NO: 73 - DNA, 22 bp, Artificial Sequence
  HY1580
gattgcctttgctcactaacct

SEQ ID NO: 74 - DNA, 23 bp, Artificial Sequence
  HY1581
ggtcgtagtttgctttctttgtt

SEQ ID NO: 75 - DNA, 22 bp, Artificial Sequence
  HY1582
cctttggatttcccagttttct

SEQ ID NO: 76 - DNA, 22 bp, Artificial Sequence
  HY1583
tggccttgaattagtctttgct

SEQ ID NO: 77 - DNA, 44 bp, Artificial Sequence
  HY1427
acgacgcatctcaaattcacagcatttaaaaaacataattattt

SEQ ID NO: 78 - DNA, 44 bp, Artificial Sequence
  HY1428
gtgaatttgagatgcgtcgtaactatttttgtatctaaaacttc

SEQ ID NO: 79 - DNA, 44 bp, Artificial Sequence
  HY1429
gtgctagagcgagaaaggttcgtgcaaacaatatccaggatatc

SEQ ID NO: 80 - DNA, 44 bp, Artificial Sequence
  HY1430
gaacctttctcgctctagcacagtatgtatcctgaactttggtt

SEQ ID NO: 81 - DNA, 22 bp, Artificial Sequence
  HY1584
agccctaagtgtgtaactggaa

SEQ ID NO: 82 - DNA, 22 bp, Artificial Sequence
  HY1585
caacaccgagtagcgtttgatt

SEQ ID NO: 83 - DNA, 42 bp, Artificial Sequence
  HY1589
cttatatgtagctttcgacatggcgggtgagcagcctctaat

SEQ ID NO: 84 - DNA, 24 bp, Artificial Sequence
  HY1573
catgtcgaaagctacatataagga

SEQ ID NO: 85 - DNA, 22 bp, Artificial Sequence
  HY1574
gcttcaaaccgctaacaatacc

SEQ ID NO: 86 - DNA, 43 bp, Artificial Sequence
  HK1294
taagtaccttgggttcccactatttataccatgggaggcgtca

SEQ ID NO: 87 - DNA, 48 bp, Artificial Sequence
  HK1295
atggtataaatagtgggaacccaaggtacttatttgaatgatacagtc

SEQ ID NO: 88 - DNA, 25 bp, Artificial Sequence
  HK1296
gctgcgcagcggaaaaggcggcgtg

SEQ ID NO: 89 - DNA, 23 bp, Artificial Sequence
  HK1297
ctttcgcctcttcgtttatgact

SEQ ID NO: 90 - DNA, 23 bp, Artificial Sequence
  HK1298
ccagttcttctgttgttggtgtt

SEQ ID NO: 91 - DNA, 23 bp, Artificial Sequence
  HK1299
atgtaagggaaataaagccaaca

SEQ ID NO: 92 - DNA, 22 bp, Artificial Sequence
  HK1300
agagggatggaaggagtgaaag

SEQ ID NO: 93 - DNA, 23 bp, Artificial Sequence
  HK1301
gaggcaatgaagaggtagagaga

SEQ ID NO: 94 - DNA, 25 bp, Artificial Sequence
  HK1302
tcagagaaatgatgaaacaagacag

SEQ ID NO: 95 - DNA, 23 bp, Artificial Sequence
  HK1303
atcactgcgtcgttaagatttgt

SEQ ID NO: 96 - DNA, 49 bp, Artificial Sequence
  HY1660
ggactatcctaagcaagcattctttagggagttacagagaataatcacc

SEQ ID NO: 97 - DNA, 23 bp, Artificial Sequence
  HY1669
agaatgcttgcttaggatagtcc

SEQ ID NO: 98 - DNA, 22 bp, Artificial Sequence
  HY1670
agatattttcgagagcgctagc

SEQ ID NO: 99 - DNA, 47 bp, Artificial Sequence
  HY1663
gctagcgctctcgaaaatatctatgattgtctcaccctgtttttggt

SEQ ID NO: 100 - DNA, 26 bp, Artificial Sequence
  HK1304
cttgcccccactcccctttctaagaa

SEQ ID NO: 101 - DNA, 49 bp, Artificial Sequence
  HK1305
gtagctttcgacatttaatgtacacacatttttaaaaaccatttgggag

SEQ ID NO: 102 - DNA, 47 bp, Artificial Sequence
  HK1306
ttttaaaaatgtgtgtacattaaatgtcgaaagctacatataaggaa

SEQ ID NO: 103 - DNA, 20 bp, Artificial Sequence
  HY2639
tcactgcccgctttccagtc

SEQ ID NO: 104 - DNA, 45 bp, Artificial Sequence
  HY2640
tgccggtgatgcggcactcgatctccctgatgcggtattttctcc

SEQ ID NO: 105 - DNA, 70 bp, Artificial Sequence
  HY2641
cgagtgccgcatcaccggcaattgacgcgtgctcaattcgataatcatattgtgacgtacgttaaagata

SEQ ID NO: 106 - DNA, 70 bp, Artificial Sequence
  HY2642
cccctcgatatacagaccgataaaacacatgcgtcaattttacacatgattatctttaacgtacgtcaca

SEQ ID NO: 107 - DNA, 45 bp, Artificial Sequence
  HY2643
tcggtctgtatatcgagggggcagagcgcacatcgcccacagtcc

SEQ ID NO: 108 - DNA, 43 bp, Artificial Sequence
  HY2644
gctggcgtgctggtggcaggggtagctggccatggtggcgata

SEQ ID NO: 109 - DNA, 44 bp, Artificial Sequence
  HY2645
gccagctacccctgccaccagcacgccagcgccttcgaccaggc

SEQ ID NO: 110 - DNA, 80 bp, Artificial Sequence
  HY2646
tcctgctgtcttctgggtctcagggcggttcttctgttgctgtggcctctgcttctggcggcctggtcgaaggcgctggc

SEQ ID NO: 111 - DNA, 80 bp, Artificial Sequence
  HY2647
agacccagaagacagcaggaggccaccgaggtgagactggagcagaagatgcccaccctgctgagagtgtacatcgacgg

SEQ ID NO: 112 - DNA, 80 bp, Artificial Sequence
  HY2648
tctctgctgcccagggccaccagcagctgggtggtggtggtcttgcccatgccgtgggggccgtcgatgtacactctcag

SEQ ID NO: 113 - DNA, 80 bp, Artificial Sequence
  HY2649
gtggccctgggcagcagagacgacatcgtgtacgtgcccgagcccatgacctactggcaggtgctgggcgccagcgagac

SEQ ID NO: 114 - DNA, 80 bp, Artificial Sequence
  HY2650
tcgccggcgctgatctcgccctggtccagtctgtgctgggtggtgtagatgttggcgatggtctcgctggcgcccagcac

SEQ ID NO: 115 - DNA, 80 bp, Artificial Sequence
  HY2651
ggcgagatcagcgccggcgacgccgccgtggtgatgaccagcgcccagatcaccatgggcatgccctacgccgtgaccga

SEQ ID NO: 116 - DNA, 80 bp, Artificial Sequence
  HY2652
gccgggggcggggcgtggctgctgccggcctcgccgcccacgtggggggccagcacggcgtcggtcacggcgtagggcat

SEQ ID NO: 117 - DNA, 80 bp, Artificial Sequence
  HY2653
agccacgccccgcccccggccctgaccatcttcctggacagacaccccatcgccttcatgctgtgctaccccgccgccag

SEQ ID NO: 118 - DNA, 80 bp, Artificial Sequence
  HY2654
ggggggatcagggccacgaaggccagcacggcctggggggtcatgctgcccatcaggtatctggcggcggggtagcacag

SEQ ID NO: 119 - DNA, 80 bp, Artificial Sequence
  HY2655
ttcgtggccctgatcccccccaccctgcccggcaccaacatcgtgctgggcgccctgcccgaggacagacacatcgacag

SEQ ID NO: 120 - DNA, 80 bp, Artificial Sequence
  HY2656
ctgatggcggccagcatggccaggtccagtctctcgccgggtctctgtctcttggccagtctgtcgatgtgtctgtcctc

SEQ ID NO: 121 - DNA, 80 bp, Artificial Sequence
  HY2657
gccatgctggccgccatcagaagagtgtacggcctgctggccaacaccgtgagatacctgcagggcggcggcagctggtg

SEQ ID NO: 122 - DNA, 80 bp, Artificial Sequence
  HY2658
ctctggggctcggcgccctgggggggcacggcggtgccgctcagctggccccagtcctcccaccagctgccgccgccctg

SEQ ID NO: 123 - DNA, 80 bp, Artificial Sequence
  HY2659
cagggcgccgagccccagagcaacgccggccccagaccccacatcggcgacaccctgttcaccctgttcagagcccccga

SEQ ID NO: 124 - DNA, 80 bp, Artificial Sequence
  HY2660
gccagcacgtccagggcccaggcgaacacgttgtacaggtcgccgttgggggccagcagctcgggggctctgaacagggt

SEQ ID NO: 125 - DNA, 80 bp, Artificial Sequence
  HY2661
tgggccctggacgtgctggccaagagactgagacccatgcacgtgttcatcctggactacgaccagagccccgccggctg

SEQ ID NO: 126 - DNA, 80 bp, Artificial Sequence
  HY2662
ccgggggtggtcacgtgggtctgcaccatgccgctggtcagctgcagcagggcgtctctgcagccggcggggctctggtc

SEQ ID NO: 127 - DNA, 44 bp, Artificial Sequence; identical to SEQ ID NO: 109
  HY2663

SEQ ID NO: 128 - DNA, 80 bp, Artificial Sequence
  HY2664
gttggcctcgcccatctctctggcgaaggttctggccaggtcgcagatggtggggatgctgccgggggtggtcacgtggg

SEQ ID NO: 129 - DNA, 40 bp, Artificial Sequence
  HY2665
gagagatgggcgaggccaacgagggcagaggaagtcttct

SEQ ID NO: 130 - DNA, 40 bp, Artificial Sequence
  HY2666
tgagtcaaaatgacgcatgagacttcgttcctgtgaggac

SEQ ID NO: 131 - DNA, 60 bp, Artificial Sequence
  HY2667
tcatgcgtcattttgactcacgcggtcgttatagttcaaaatcagtgacacttaccgcat

SEQ ID NO: 132 - DNA, 60 bp, Artificial Sequence
  HY2668
ggaaagcgggcagtgaagctcccgtgaggcgtgcttgtcaatgcggtaagtgtcactgat

SEQ ID NO: 133 - DNA, 22 bp, Artificial Sequence
  1st STEP forward for L1-R1
tggtaaggatgagggaaagatg

SEQ ID NO: 134 - DNA, 21 bp, Artificial Sequence
  1st STEP reverse for L1-R1
gccaagtagcaaagagcgtgt

SEQ ID NO: 135 - DNA, 24 bp, Artificial Sequence
  2nd STEP forward for L1-R1
atataagaaggacgaggagaaatg

SEQ ID NO: 136 - DNA, 21 bp, Artificial Sequence
  2nd STEP reverse for L1-R1
ggccaatatgtgctttaggaa

SEQ ID NO: 137 - DNA, 24 bp, Artificial Sequence
  1st STEP forward for L2-R1
tggcatatttgttaatgttctgct

SEQ ID NO: 138 - DNA, 21 bp, Artificial Sequence
  1st STEP reverse for L2-R1
gccaagtagcaaagagcgtgt

SEQ ID NO: 139 - DNA, 23 bp, Artificial Sequence
  2nd STEP forward for L2-R1
ataagaccaacttcagacaccag

SEQ ID NO: 140 - DNA, 21 bp, Artificial Sequence
  2nd STEP reverse for L2-R1
ggccaatatgtgctttaggaa

SEQ ID NO: 141 - DNA, 22 bp, Artificial Sequence
  1st STEP forward for L3-R1
aaagagatcatggggtagcaaa

SEQ ID NO: 142 - DNA, 21 bp, Artificial Sequence
  1st STEP reverse for L3-R1
gccaagtagcaaagagcgtgt

SEQ ID NO: 143 - DNA, 21 bp, Artificial Sequence
  2nd STEP forward for L3-R1
gtagccaagagggctgagagt

SEQ ID NO: 144 - DNA, 21 bp, Artificial Sequence
  2nd STEP reverse for L3-R1
ggccaatatgtgctttaggaa

SEQ ID NO: 145 - DNA, 21 bp, Artificial Sequence
  1st STEP forward for L4-R1
cagacttggatgtggaccttg

SEQ ID NO: 146 - DNA, 21 bp, Artificial Sequence
  1st STEP reverse for L4-R1
gccaagtagcaaagagcgtgt

SEQ ID NO: 147 - DNA, 24 bp, Artificial Sequence
  2nd STEP forward for L4-R1
gatcatagcaaaagctcagttgtc

SEQ ID NO: 148 - DNA, 21 bp, Artificial Sequence
  2nd STEP reverse for L4-R1
ggccaatatgtgctttaggaa

SEQ ID NO: 149 - DNA, 21 bp, Artificial Sequence
  1st STEP forward for L5-R1
cccatcctgtgcttcttctct

SEQ ID NO: 150 - DNA, 21 bp, Artificial Sequence
  1st STEP reverse for L5-R1
gccaagtagcaaagagcgtgt

SEQ ID NO: 151 - DNA, 21 bp, Artificial Sequence
  2nd STEP forward for L5-R1
gcactcatgtgctctggtctt

SEQ ID NO: 152 - DNA, 21 bp, Artificial Sequence
  2nd STEP reverse for L5-R1
ggccaatatgtgctttaggaa

SEQ ID NO: 153 - DNA, 21 bp, Artificial Sequence
  1st STEP forward for L4-R2
cagacttggatgtggaccttg

SEQ ID NO: 154 - DNA, 20 bp, Artificial Sequence
  1st STEP reverse for L4-R2
tcctgaaccacaccttggac

SEQ ID NO: 155 - DNA, 24 bp, Artificial Sequence
  2nd STEP forward for L4-R2
gatcatagcaaaagctcagttgtc

SEQ ID NO: 156 - DNA, 22 bp, Artificial Sequence
  2nd STEP reverse for L4-R2
acgagaggcagctctattcatc

SEQ ID NO: 157 - DNA, 21 bp, Artificial Sequence
  1st STEP forward for L4-R3
cagacttggatgtggaccttg

SEQ ID NO: 158 - DNA, 25 bp, Artificial Sequence
  1st STEP reverse for L4-R3
ttgtaacctgtgttttcatgttttt

SEQ ID NO: 159 - DNA, 24 bp, Artificial Sequence
  2nd STEP forward for L4-R3
gatcatagcaaaagctcagttgtc

SEQ ID NO: 160 - DNA, 22 bp, Artificial Sequence
  2nd STEP reverse for L4-R3
tggcacaaaggagagaataaca

SEQ ID NO: 161 - DNA, 21 bp, Artificial Sequence
  1st STEP forward for L4-R4
cagacttggatgtggaccttg

SEQ ID NO: 162 - DNA, 22 bp, Artificial Sequence
  1st STEP reverse for L4-R4
gcttgctaggattttggttttt

SEQ ID NO: 163 - DNA, 24 bp, Artificial Sequence
  2nd STEP forward for L4-R4
gatcatagcaaaagctcagttgtc

SEQ ID NO: 164 - DNA, 24 bp, Artificial Sequence
  2nd STEP reverse for L4-R4
ccacagattcattaaaaggaggag

SEQ ID NO: 165 - DNA, 21 bp, Artificial Sequence
  1st STEP forward for L4-R5
cagacttggatgtggaccttg

SEQ ID NO: 166 - DNA, 22 bp, Artificial Sequence
  1st STEP reverse for L4-R5
cacttctggggtcacttaggaa

SEQ ID NO: 167 - DNA, 24 bp, Artificial Sequence
  2nd STEP forward for L4-R5
gatcatagcaaaagctcagttgtc

SEQ ID NO: 168 - DNA, 22 bp, Artificial Sequence
  2nd STEP reverse for L4-R5
ctagctgtaccttgcacctttg

SEQ ID NO: 169 - DNA, 21 bp, Artificial Sequence
  1st STEP forward for L4-R6
cagacttggatgtggaccttg

SEQ ID NO: 170 - DNA, 23 bp, Artificial Sequence
  1st STEP reverse for L4-R6
ccaaggtaccacttaatgcttca

SEQ ID NO: 171 - DNA, 24 bp, Artificial Sequence
  2nd STEP forward for L4-R6
gatcatagcaaaagctcagttgtc

SEQ ID NO: 172 - DNA, 23 bp, Artificial Sequence
  2nd STEP reverse for L4-R6
tactcggcaggtagtaaacttct

SEQ ID NO: 173 - DNA, 20 bp, Artificial Sequence
  1st STEP forward for L6-R1
ctccctggcttttgtgttgg

SEQ ID NO: 174 - DNA, 21 bp, Artificial Sequence
  1st STEP reverse for L6-R1
gccaagtagcaaagagcgtgt

SEQ ID NO: 175 - DNA, 20 bp, Artificial Sequence
  2nd STEP forward for L6-R1
ctccctggcttttgtgttgg

SEQ ID NO: 176 - DNA, 21 bp, Artificial Sequence
  2nd STEP reverse for L6-R1
ggccaatatgtgctttaggaa

SEQ ID NO: 177 - DNA, 25 bp, Artificial Sequence
  1st STEP forward for L7-R1
caccgaccagaccctgggatcgtcc

SEQ ID NO: 178 - DNA, 21 bp, Artificial Sequence
  1st STEP reverse for L7-R1
gccaagtagcaaagagcgtgt

SEQ ID NO: 179 - DNA, 22 bp, Artificial Sequence
  2nd STEP forward for L7-R1
ctgtggagattagtcagcccaa

SEQ ID NO: 180 - DNA, 21 bp, Artificial Sequence
  2nd STEP reverse for L7-R1
ggccaatatgtgctttaggaa

SEQ ID NO: 181 - DNA, 21 bp, Artificial Sequence
  1st STEP forward for L4-R7
cagacttggatgtggaccttg

SEQ ID NO: 182 - DNA, 22 bp, Artificial Sequence
  1st STEP reverse for L4-R7
ctgctggacgttttggtaatgc

SEQ ID NO: 183 - DNA, 24 bp, Artificial Sequence
  2nd STEP forward for L4-R7
gatcatagcaaaagctcagttgtc

SEQ ID NO: 184 - DNA, 21 bp, Artificial Sequence
  2nd STEP reverse for L4-R7
ccagctatccacgccatttag

SEQ ID NO: 185 - DNA, 21 bp, Artificial Sequence
  1st STEP forward for L4-R8
cagacttggatgtggaccttg

SEQ ID NO: 186 - DNA, 23 bp, Artificial Sequence
  1st STEP reverse for L4-R8
ggaagaaggcaaatcaaaaggtc

SEQ ID NO: 187 - DNA, 24 bp, Artificial Sequence
  2nd STEP forward for L4-R8
gatcatagcaaaagctcagttgtc

SEQ ID NO: 188 - DNA, 25 bp, Artificial Sequence
  2nd STEP reverse for L4-R8
gcttgactcttctaattctcactgc

SEQ ID NO: 189 - DNA, 22 bp, Artificial Sequence
  1st STEP forward for L8-R9
tttgtggttctggcatattggg

SEQ ID NO: 190 - DNA, 22 bp, Artificial Sequence
  1st STEP reverse for L8-R9
atgcctccttgacttccatcag

SEQ ID NO: 191 - DNA, 22 bp, Artificial Sequence
  2nd STEP forward for L8-R9
aaaagcaaagcagaattccgga

SEQ ID NO: 192 - DNA, 22 bp, Artificial Sequence
  2nd STEP reverse for L8-R9
taaagtgacgagcaagcaagga

SEQ ID NO: 193 - DNA, 22 bp, Artificial Sequence
  1st STEP forward for L9-R9
taattgaagaagccctcgaccc

SEQ ID NO: 194 - DNA, 22 bp, Artificial Sequence
  1st STEP reverse for L9-R9
atgcctccttgacttccatcag

SEQ ID NO: 195 - DNA, 22 bp, Artificial Sequence
  2nd STEP forward for L9-R9
accccttttactatccacaggc

SEQ ID NO: 196 - DNA, 22 bp, Artificial Sequence
  2nd STEP reverse for L9-R9
taaagtgacgagcaagcaagga

SEQ ID NO: 197 - DNA, 22 bp, Artificial Sequence
  1st STEP forward for L10-R9
atgattgtcccagtctttcccc

SEQ ID NO: 198 - DNA, 22 bp, Artificial Sequence
  1st STEP reverse for L10-R9
atgcctccttgacttccatcag

SEQ ID NO: 199 - DNA, 22 bp, Artificial Sequence
  2nd STEP forward for L10-R9
acagggaagttgcaaagacaaa

SEQ ID NO: 200 - DNA, 22 bp, Artificial Sequence
  2nd STEP reverse for L10-R9
taaagtgacgagcaagcaagga

SEQ ID NO: 201 - DNA, 23 bp, Artificial Sequence
  1st STEP forward for L11-R9
aggcagttaaggaaaagtaccca

SEQ ID NO: 202 - DNA, 22 bp, Artificial Sequence
  1st STEP reverse for L11-R9
atgcctccttgacttccatcag

SEQ ID NO: 203 - DNA, 22 bp, Artificial Sequence
  2nd STEP forward for L11-R9
tctgatctattcctgggctggt

SEQ ID NO: 204 - DNA, 22 bp, Artificial Sequence
  2nd STEP reverse for L11-R9
taaagtgacgagcaagcaagga

SEQ ID NO: 205 - DNA, 21 bp, Artificial Sequence
  1st STEP forward for L12-R9
aaataaggctgggcatggttg

SEQ ID NO: 206 - DNA, 22 bp, Artificial Sequence
  1st STEP reverse for L12-R9
atgcctccttgacttccatcag

SEQ ID NO: 207 - DNA, 22 bp, Artificial Sequence
  2nd STEP forward for L12-R9
gcaaaccaaaaccacgagatac

SEQ ID NO: 208 - DNA, 22 bp, Artificial Sequence
  2nd STEP reverse for L12-R9
taaagtgacgagcaagcaagga

SEQ ID NO: 209 - DNA, 22 bp, Artificial Sequence
  1st STEP forward for GPR119
gcccttaccgtcttagccatca

SEQ ID NO: 210 - DNA, 22 bp, Artificial Sequence
  1st STEP reverse for GPR119
cgacatgctcaagattgcctcc

SEQ ID NO: 211 - DNA, 22 bp, Artificial Sequence
  2nd STEP forward for GPR119
ctgctgatctagttggggctcc

SEQ ID NO: 212 - DNA, 23 bp, Artificial Sequence
  2nd STEP reverse for GPR119
gctgtatttcaccctcacttcgt

SEQ ID NO: 213 - DNA, 22 bp, Artificial Sequence
  1st STEP forward for RBMX2
cactgaagcatcgcctgtcttg

SEQ ID NO: 214 - DNA, 22 bp, Artificial Sequence
  1st STEP reverse for RBMX2
atgtcgagtggctgtacaaggt

SEQ ID NO: 215 - DNA, 22 bp, Artificial Sequence
  2nd STEP forward for RBMX2
tcactgaagcatcgcctgtctt

SEQ ID NO: 216 - DNA, 21 bp, Artificial Sequence
  2nd STEP reverse for RBMX2
ggagaacaaccttggcagcag

SEQ ID NO: 217 - DNA, 22 bp, Artificial Sequence
  1st STEP forward for DENND10P1
gaaaggtcccaagtcaaaggaa

SEQ ID NO: 218 - DNA, 20 bp, Artificial Sequence
  1st STEP reverse for DENND10P1
gggtcagaaaccacaccaag

SEQ ID NO: 219 - DNA, 22 bp, Artificial Sequence
  2nd STEP forward for DENND10P1
ccagccctacatgtgttcagga

SEQ ID NO: 220 - DNA, 22 bp, Artificial Sequence
  2nd STEP reverse for DENND10P1
ccgccacaaccccatatgtaga

SEQ ID NO: 221 - DNA, 22 bp, Artificial Sequence
  1st STEP forward for ENOX2,LOC105373338
aagccagttttcagcacgaatg

SEQ ID NO: 222 - DNA, 22 bp, Artificial Sequence
  1st STEP reverse for ENOX2,LOC105373338
aacagagaggatggaggtttgg

SEQ ID NO: 223 - DNA, 22 bp, Artificial Sequence
  2nd STEP forward for ENOX2,LOC105373338
ccaagagcccgagactgatgaa

SEQ ID NO: 224 - DNA, 22 bp, Artificial Sequence
  2nd STEP reverse for ENOX2,LOC105373338
ttcccctctggccttcttacag

SEQ ID NO: 225 - DNA, 22 bp, Artificial Sequence
  1st STEP forward for LINC01201,ARHGAP36
tcctctagaacggaccagtgat

SEQ ID NO: 226 - DNA, 21 bp, Artificial Sequence
  1st STEP reverse for LINC01201,ARHGAP36
cgaagggaggcagagacacac

SEQ ID NO: 227 - DNA, 22 bp, Artificial Sequence
  2nd STEP forward for LINC01201,ARHGAP36
tcctgctcacattcttggtcct

SEQ ID NO: 228 - DNA, 22 bp, Artificial Sequence
  2nd STEP reverse for LINC01201,ARHGAP36
acccagctaagagtgtttcggt

SEQ ID NO: 229 - DNA, 22 bp, Artificial Sequence
  1st STEP forward for IGSF1
acattacacccaggaagagcgg

SEQ ID NO: 230 - DNA, 22 bp, Artificial Sequence
  1st STEP reverse for IGSF1
aggtgcccttactgagtccaat

SEQ ID NO: 231 - DNA, 22 bp, Artificial Sequence
  2nd STEP forward for IGSF1
tggatatgagtgcggcagatgt

SEQ ID NO: 232 - DNA, 22 bp, Artificial Sequence
  2nd STEP reverse for IGSF1
ggatctgggtccgggctaattt

SEQ ID NO: 233 - DNA, 22 bp, Artificial Sequence
  1st STEP forward for OR13H1
tcaaacgagtgtctccttggct

SEQ ID NO: 234 - DNA, 22 bp, Artificial Sequence
  1st STEP reverse for OR13H1
tcagggtaggacttggactgag

SEQ ID NO: 235 - DNA, 24 bp, Artificial Sequence
  2nd STEP forward for OR13H1
aatttacctcagcacattgttggg

SEQ ID NO: 236 - DNA, 25 bp, Artificial Sequence
  2nd STEP reverse for OR13H1
caacataactttccttattgcccgt

SEQ ID NO: 237 - DNA, 24 bp, Artificial Sequence
  1st STEP forward for FIRRE
cactgttggcaccgtttagatttt

SEQ ID NO: 238 - DNA, 22 bp, Artificial Sequence
  1st STEP reverse for FIRRE
tgaccacgcacaaacagatgag

SEQ ID NO: 239 - DNA, 23 bp, Artificial Sequence
  2nd STEP forward for FIRRE
tgcacaaattcttcaacaccacc

SEQ ID NO: 240 - DNA, 21 bp, Artificial Sequence
  2nd STEP reverse for FIRRE
gtattcgtctctctccccgcc

SEQ ID NO: 241 - DNA, 22 bp, Artificial Sequence
  1st STEP forward for MST4
ggggtgtggtatgggacttcaa

SEQ ID NO: 242 - DNA, 22 bp, Artificial Sequence
  1st STEP reverse for MST4
cccctttcctccatcctagcac

SEQ ID NO: 243 - DNA, 24 bp, Artificial Sequence
  2nd STEP forward for MST4
tctaggtgaagcatactccagtgt

SEQ ID NO: 244 - DNA, 24 bp, Artificial Sequence
  2nd STEP reverse for MST4
aggaggcaattctataggcaagct

SEQ ID NO: 245 - DNA, 24 bp, Artificial Sequence
  1st STEP forward for FRMD7
cgctattctccctcctgttacaca

SEQ ID NO: 246 - DNA, 22 bp, Artificial Sequence
  1st STEP reverse for FRMD7
tgtttacgtgtggcagtgttgt

SEQ ID NO: 247 - DNA, 22 bp, Artificial Sequence
  2nd STEP forward for FRMD7
aagccctcattgtcacgatgtt

SEQ ID NO: 248 - DNA, 22 bp, Artificial Sequence
  2nd STEP reverse for FRMD7
acctcgtaccagtgcttcatcc

SEQ ID NO: 249 - DNA, 22 bp, Artificial Sequence
  1st STEP forward for RAP2C,RAP2C-AS1,MBNL3
ttcaccctgactgacttttgct

SEQ ID NO: 250 - DNA, 23 bp, Artificial Sequence
  1st STEP reverse for RAP2C,RAP2C-AS1,MBNL3
tgggactgacatttaaaacgcct

SEQ ID NO: 251 - DNA, 23 bp, Artificial Sequence
  2nd STEP forward for RAP2C,RAP2C-AS1,MBNL3
acgaaactcagttgaaccgaagc

SEQ ID NO: 252 - DNA, 25 bp, Artificial Sequence
  2nd STEP reverse for RAP2C,RAP2C-AS1,MBNL3
agtggggaacagaagtatatgtgct

SEQ ID NO: 253 - DNA, 22 bp, Artificial Sequence
  1st STEP forward for HS6ST2,HS6ST2-AS1
gtgagtctggtttggctttcgg

SEQ ID NO: 254 - DNA, 22 bp, Artificial Sequence
  1st STEP reverse for HS6ST2,HS6ST2-AS1
tcagacccatttccagagccag

SEQ ID NO: 255 - DNA, 24 bp, Artificial Sequence
  2nd STEP forward for HS6ST2,HS6ST2-AS1
ttctacagctcggtaagattcacc

SEQ ID NO: 256 - DNA, 22 bp, Artificial Sequence
  2nd STEP reverse for HS6ST2,HS6ST2-AS1
acaacctctctgtcatgcctga

SEQ ID NO: 257 - DNA, 22 bp, Artificial Sequence
  1st STEP forward for USP26
aacgcctatcctcctgcatctg

SEQ ID NO: 258 - DNA, 22 bp, Artificial Sequence
  1st STEP reverse for USP26
actcagcagtgtgacggtatga

SEQ ID NO: 259 - DNA, 23 bp, Artificial Sequence
  2nd STEP forward for USP26
agctatgggattgaggtgtctgt

SEQ ID NO: 260 - DNA, 22 bp, Artificial Sequence
  2nd STEP reverse for USP26
tcaaacagtgcccgaaaatcca

SEQ ID NO: 261 - DNA, 22 bp, Artificial Sequence
  1st STEP forward for TFDP3
cccaaaagtcatgcccatccac

SEQ ID NO: 262 - DNA, 22 bp, Artificial Sequence
  1st STEP reverse for TFDP3
cctgtgccgtctttccatgaag

SEQ ID NO: 263 - DNA, 22 bp, Artificial Sequence
  2nd STEP forward for TFDP3
tcgcaatgttggtcaggtcact

SEQ ID NO: 264 - DNA, 22 bp, Artificial Sequence
  2nd STEP reverse for TFDP3
gcctctcagaaccagcattcct

SEQ ID NO: 265 - DNA, 22 bp, Artificial Sequence
  1st STEP forward for GPC4
ttgcccgagtgttgacagctat

SEQ ID NO: 266 - DNA, 22 bp, Artificial Sequence
  1st STEP reverse for GPC4
tctggagagacgtggaggtgat

SEQ ID NO: 267 - DNA, 22 bp, Artificial Sequence
  2nd STEP forward for GPC4
tctggacacctagttctcccct

SEQ ID NO: 268 - DNA, 22 bp, Artificial Sequence
  2nd STEP reverse for GPC4
aagcaaaccagggtcccttctt

SEQ ID NO: 269 - DNA, 22 bp, Artificial Sequence
  1st STEP forward for GPC3,GPC3-AS1
cagggaggtgggtttcaaggaa

SEQ ID NO: 270 - DNA, 22 bp, Artificial Sequence
  1st STEP reverse for GPC3,GPC3-AS1
gtgtgcttcttcttcctggtgc

SEQ ID NO: 271 - DNA, 25 bp, Artificial Sequence
  2nd STEP forward for GPC3,GPC3-AS1
agttgtaaagagagaccagaccagg

SEQ ID NO: 272 - DNA, 23 bp, Artificial Sequence
  2nd STEP reverse for GPC3,GPC3-AS1
actggcctatgatctggatgtgg

SEQ ID NO: 273 - DNA, 22 bp, Artificial Sequence
  1st STEP forward for microRNAs
atcctcctttcttccacaggcc

SEQ ID NO: 274 - DNA, 22 bp, Artificial Sequence
  1st STEP reverse for microRNAs
actgccctaaatgccccttctg

SEQ ID NO: 275 - DNA, 22 bp, Artificial Sequence
  2nd STEP forward for microRNAs
gctgatcaggaatgtcgccaac

SEQ ID NO: 276 - DNA, 22 bp, Artificial Sequence
  2nd STEP reverse for microRNAs
aggccttggccatgtaaaagtg

SEQ ID NO: 277 - DNA, 22 bp, Artificial Sequence
  1st STEP forward for CCDC160
cagatagcagcaagggaatgga

SEQ ID NO: 278 - DNA, 22 bp, Artificial Sequence
  1st STEP reverse for CCDC160
tgacttctttggcttgctggag

SEQ ID NO: 279 - DNA, 24 bp, Artificial Sequence
  2nd STEP forward for CCDC160
cagatattggaagaggtgcctgga

SEQ ID NO: 280 - DNA, 21 bp, Artificial Sequence
  2nd STEP reverse for CCDC160
gagcacatttccaacctcggt

SEQ ID NO: 281 - DNA, 22 bp, Artificial Sequence
  1st STEP forward for PHF6
gggttaccgcttgctaaggact

SEQ ID NO: 282 - DNA, 23 bp, Artificial Sequence
  1st STEP reverse for PHF6
tggtactgaggtgctatggtagt

SEQ ID NO: 283 - DNA, 22 bp, Artificial Sequence
  2nd STEP forward for PHF6
cttgacagcacacctcctctct

SEQ ID NO: 284 - DNA, 25 bp, Artificial Sequence
  2nd STEP reverse for PHF6
acttgacaaacgtgatcttaaggga

SEQ ID NO: 285 - DNA, 23 bp, Artificial Sequence
  1st STEP forward for HPRT1
cctttgggcggattgttgtttaa

SEQ ID NO: 286 - DNA, 22 bp, Artificial Sequence
  1st STEP reverse for HPRT1
tttgtagctccgccaacccatt

SEQ ID NO: 287 - DNA, 25 bp, Artificial Sequence
  2nd STEP forward for HPRT1
actggaaaagcaaaatacaaagcct

SEQ ID NO: 288 - DNA, 23 bp, Artificial Sequence
  2nd STEP reverse for HPRT1
ggaacacgtgtaagctagatggc

SEQ ID NO: 289 - DNA, 22 bp, Artificial Sequence
  1st STEP forward for microRNAs-2
ccttatgtcaggggttcatgct

SEQ ID NO: 290 - DNA, 22 bp, Artificial Sequence
  1st STEP reverse for microRNAs-2
tggggaaaagaggctatcagga

SEQ ID NO: 291 - DNA, 20 bp, Artificial Sequence
  2nd STEP forward for microRNAs-2
caatgcgtcttgaggccctg

SEQ ID NO: 292 - DNA, 25 bp, Artificial Sequence
  2nd STEP reverse for microRNAs-2
tctgagttgtggtataaaggtgacc

SEQ ID NO: 293 - DNA, 23 bp, Artificial Sequence
  1st STEP forward for MIR503HG,microRNAs
tggaggaaaatctaggcacactg

SEQ ID NO: 294 - DNA, 22 bp, Artificial Sequence
  1st STEP reverse for MIR503HG,microRNAs
gaaatccccattctgctcccgc

SEQ ID NO: 295 - DNA, 22 bp, Artificial Sequence
  2nd STEP forward for MIR503HG,microRNAs
agtttaagggccacgtctgtct

SEQ ID NO: 296 - DNA, 22 bp, Artificial Sequence
  2nd STEP reverse for MIR503HG,microRNAs
ggcccctagaagtttcccagtt

SEQ ID NO: 297 - DNA, 22 bp, Artificial Sequence
  1st STEP forward for LINC00629
ttcatgttcccaggtggcaagg

SEQ ID NO: 298 - DNA, 22 bp, Artificial Sequence
  1st STEP reverse for LINC00629
catccaaggacaagaggcaggg

SEQ ID NO: 299 - DNA, 23 bp, Artificial Sequence
  2nd STEP forward for LINC00629
actcgattctctccctacactgg

SEQ ID NO: 300 - DNA, 22 bp, Artificial Sequence
  2nd STEP reverse for LINC00629
tttcaaagtggggtgaggaggt

SEQ ID NO: 301 - DNA, 22 bp, Artificial Sequence
  1st STEP forward for PLAC1
agggacctgggtatgctcttct

SEQ ID NO: 302 - DNA, 22 bp, Artificial Sequence
  1st STEP reverse for PLAC1
gatcctcctcacctctgcgttt

SEQ ID NO: 303 - DNA, 25 bp, Artificial Sequence
  2nd STEP forward for PLAC1
ggacccaatcatatcatctgtgtga

SEQ ID NO: 304 - DNA, 25 bp, Artificial Sequence
  2nd STEP reverse for PLAC1
gttctgttttgggttcatcttgagg

SEQ ID NO: 305 - DNA, 22 bp, Artificial Sequence
  1st STEP forward for FAM122B,FAM122C
ggcaaccacaaaccccaaatct

SEQ ID NO: 306 - DNA, 22 bp, Artificial Sequence
  1st STEP reverse for FAM122B,FAM122C
ggtggctgggagtagaagtagc

SEQ ID NO: 307 - DNA, 22 bp, Artificial Sequence
  2nd STEP forward for FAM122B,FAM122C
agttgccatgcctgttcctttc

SEQ ID NO: 308 - DNA, 25 bp, Artificial Sequence
  2nd STEP reverse for FAM122B,FAM122C
cccaaattaagtactacaagtggcg

SEQ ID NO: 309 - DNA, 20 bp, Artificial Sequence
  1st STEP forward for MOSPD1
gcagggaggggcttggaaga

SEQ ID NO: 310 - DNA, 24 bp, Artificial Sequence
  1st STEP reverse for MOSPD1
cactttgattgctaggggtcatgt

SEQ ID NO: 311 - DNA, 22 bp, Artificial Sequence
  2nd STEP forward for MOSPD1
tgacttaggctcctcacatggt

SEQ ID NO: 312 - DNA, 22 bp, Artificial Sequence
  2nd STEP reverse for MOSPD1
aggatgcttctgagtgacacct

SEQ ID NO: 313 - DNA, 22 bp, Artificial Sequence
  1st STEP forward for LINC02243
ccactggcatttctaccaccca

SEQ ID NO: 314 - DNA, 22 bp, Artificial Sequence
  1st STEP reverse for LINC02243
cagcacagcagttccatgtcac

SEQ ID NO: 315 - DNA, 22 bp, Artificial Sequence
  2nd STEP forward for LINC02243
ccccagtcccattatctgcctt

SEQ ID NO: 316 - DNA, 22 bp, Artificial Sequence
  2nd STEP reverse for LINC02243
tgcatcgtcacaggcagtaaga

SEQ ID NO: 317 - DNA, 22 bp, Artificial Sequence
  1st STEP forward for SMIM10
tgattctcaacgtccacctgca

SEQ ID NO: 318 - DNA, 22 bp, Artificial Sequence
  1st STEP reverse for SMIM10
gggagatttgcctgctgtctga

SEQ ID NO: 319 - DNA, 20 bp, Artificial Sequence
  2nd STEP forward for SMIM10
catccctctgtcccacggtc

SEQ ID NO: 320 - DNA, 23 bp, Artificial Sequence
  2nd STEP reverse for SMIM10
caactgttcaaaaccatgccaca

SEQ ID NO: 321 - DNA, 22 bp, Artificial Sequence
  1st STEP forward for RLT8B
cctgctggctgacttctcacat

SEQ ID NO: 322 - DNA, 22 bp, Artificial Sequence
  1st STEP reverse for RLT8B
ctgttaccttcagcgagaccca

SEQ ID NO: 323 - DNA, 25 bp, Artificial Sequence
  2nd STEP forward for RLT8B
cagctgttcaccaataatctgtgtg

SEQ ID NO: 324 - DNA, 22 bp, Artificial Sequence
  2nd STEP reverse for RLT8B
agacgactacatcatgctgccc

SEQ ID NO: 325 - DNA, 22 bp, Artificial Sequence
  1st STEP forward for RLT8C
ctttctggccgagatgaagcga

SEQ ID NO: 326 - DNA, 20 bp, Artificial Sequence
  1st STEP reverse for RLT8C
tctgtcggtgggatgcgatg

SEQ ID NO: 327 - DNA, 21 bp, Artificial Sequence
  2nd STEP forward for RLT8C
tgcagctgataaaggccctcc

SEQ ID NO: 328 - DNA, 20 bp, Artificial Sequence
  2nd STEP reverse for RLT8C
ccagcccagatacctccgag

SEQ ID NO: 329 - DNA, 21 bp, Artificial Sequence
  1st STEP forward for RLT8A
agtctggaggagtggaggtgg

SEQ ID NO: 330 - DNA, 20 bp, Artificial Sequence
  1st STEP reverse for RLT8A
tctccaacgacgccctgaag

SEQ ID NO: 331 - DNA, 22 bp, Artificial Sequence
  2nd STEP forward for RLT8A
ctctggggatggggaggaaatg

SEQ ID NO: 332 - DNA, 22 bp, Artificial Sequence
  2nd STEP reverse for RLT8A
ttccctttcccgagacgtttga

SEQ ID NO: 333 - DNA, 22 bp, Artificial Sequence
  1st STEP forward for SMIM0L2B
aaatggggatagcaggtgaggg

SEQ ID NO: 334 - DNA, 22 bp, Artificial Sequence
  1st STEP reverse for SMIM0L2B
gggaatctggggatctcgcttt

SEQ ID NO: 335 - DNA, 22 bp, Artificial Sequence
  2nd STEP forward for SMIM0L2B
caaggtcaggggttctcaggag

SEQ ID NO: 336 - DNA, 22 bp, Artificial Sequence
  2nd STEP reverse for SMIM0L2B
tgacagaggaaaccgaggcttc

SEQ ID NO: 337 - DNA, 22 bp, Artificial Sequence
  1st STEP forward for ETDB,SMIM10L2B-AS1
cccaagtgacagagaggtgaga

SEQ ID NO: 338 - DNA, 22 bp, Artificial Sequence
  1st STEP reverse for ETDB,SMIM10L2B-AS1
gccagggtagttgagggttctg

SEQ ID NO: 339 - DNA, 22 bp, Artificial Sequence
  2nd STEP forward for ETDB,SMIM10L2B-AS1
tgggaacgtaatcacagtggct

SEQ ID NO: 340 - DNA, 22 bp, Artificial Sequence
  2nd STEP reverse for ETDB,SMIM10L2B-AS1
catggcggacaaagttgctgat

SEQ ID NO: 341 - DNA, 22 bp, Artificial Sequence
  1st STEP forward for CT55
aggggttctctgccttcctttg

SEQ ID NO: 342 - DNA, 22 bp, Artificial Sequence
  1st STEP reverse for CT55
ttcctctgtgtgtccccttgtc

SEQ ID NO: 343 - DNA, 24 bp, Artificial Sequence
  2nd STEP forward for CT55
tcaccaacatgatgagtagcacct

SEQ ID NO: 344 - DNA, 20 bp, Artificial Sequence
  2nd STEP reverse for CT55
ggtcccatgccacagtgtct

SEQ ID NO: 345 - DNA, 20 bp, Artificial Sequence
  1st STEP forward for ZNF75D,ETDA,ETDC,ZNF449
cagctcctgtccccgtttcg

SEQ ID NO: 346 - DNA, 22 bp, Artificial Sequence
  1st STEP reverse for ZNF75D,ETDA,ETDC,ZNF449
tgacgcattgaatctcacagga

SEQ ID NO: 347 - DNA, 22 bp, Artificial Sequence
  2nd STEP forward for ZNF75D,ETDA,ETDC,ZNF449
gtttcaagttccagccggtgag

SEQ ID NO: 348 - DNA, 22 bp, Artificial Sequence
  2nd STEP reverse for ZNF75D,ETDA,ETDC,ZNF449
tgagccttggagtaactggagc

SEQ ID NO: 349 - DNA, 22 bp, Artificial Sequence
  1st STEP forward for LOC100506790
tgtttggtaatcaggggagggt

SEQ ID NO: 350 - DNA, 22 bp, Artificial Sequence
  1st STEP reverse for LOC100506790
agctgccttcttctcacctctg

SEQ ID NO: 351 - DNA, 22 bp, Artificial Sequence
  2nd STEP forward for LOC100506790
accctattgagtcctgaacccg

SEQ ID NO: 352 - DNA, 22 bp, Artificial Sequence
  2nd STEP reverse for LOC100506790
tcacacatggggctgtatagga

SEQ ID NO: 353 - DNA, 22 bp, Artificial Sequence
  1st STEP forward for SMIM10L2A
atctgctcctgtccctgctttt

SEQ ID NO: 354 - DNA, 22 bp, Artificial Sequence
  1st STEP reverse for SMIM10L2A
gtccaggtcaagtcggttctca

SEQ ID NO: 355 - DNA, 22 bp, Artificial Sequence
  2nd STEP forward for SMIM10L2A
cagatgtggccctttcaaaccc

SEQ ID NO: 356 - DNA, 22 bp, Artificial Sequence
  2nd STEP reverse for SMIM10L2A
agaacaagcagctacctctcgg

SEQ ID NO: 357 - DNA, 22 bp, Artificial Sequence
  1st STEP forward for INTS6L,ISTN6L-AS1
tccctcccctagtcctgtcatc

SEQ ID NO: 358 - DNA, 22 bp, Artificial Sequence
  1st STEP reverse for INTS6L,ISTN6L-AS1
gttcatagaggcggacgtgtct

SEQ ID NO: 359 - DNA, 23 bp, Artificial Sequence
  2nd STEP forward for INTS6L,ISTN6L-AS1
cattcgaactgcttccaagtcct

SEQ ID NO: 360 - DNA, 20 bp, Artificial Sequence
  2nd STEP reverse for INTS6L,ISTN6L-AS1
ggggtcgcgtaggaaaggag

SEQ ID NO: 361 - DNA, 22 bp, Artificial Sequence
  1st STEP forward for SAGEP2
gcgagactaattgagccctcct

SEQ ID NO: 362 - DNA, 22 bp, Artificial Sequence
  1st STEP reverse for SAGEP2
ccactccattccctacccttgg

SEQ ID NO: 363 - DNA, 23 bp, Artificial Sequence
  2nd STEP forward for SAGEP2
gtatgttttgtcccatcctcccc

SEQ ID NO: 364 - DNA, 22 bp, Artificial Sequence
  2nd STEP reverse for SAGEP2
taacgcgggtcccatccatttc

SEQ ID NO: 365 - DNA, 22 bp, Artificial Sequence
  1st STEP forward for CT45A1,2,3,5,6,7,8,9,10
cctgagtcccaccataggctta

SEQ ID NO: 366 - DNA, 22 bp, Artificial Sequence
  1st STEP reverse for CT45A1,2,3,5,6,7,8,9,10
cgccacaacttcactgccattt

SEQ ID NO: 367 - DNA, 22 bp, Artificial Sequence
  2nd STEP forward for CT45A1,2,3,5,6,7,8,9,10
gcacatttcccacaactcccag

SEQ ID NO: 368 - DNA, 22 bp, Artificial Sequence
  2nd STEP reverse for CT45A1,2,3,5,6,7,8,9,10
agacagagttcccaaggtcacg

SEQ ID NO: 369 - DNA, 22 bp, Artificial Sequence
  1st STEP forward for SAGE1
gtctttggtggaaactgtgcca

SEQ ID NO: 370 - DNA, 22 bp, Artificial Sequence
  1st STEP reverse for SAGE1
cactcaccttgctgcttccttg

SEQ ID NO: 371 - DNA, 22 bp, Artificial Sequence
  2nd STEP forward for SAGE1
acaggacattgtatgccaccca

SEQ ID NO: 372 - DNA, 22 bp, Artificial Sequence
  2nd STEP reverse for SAGE1
ggccagggattaggaggaacaa

SEQ ID NO: 373 - DNA, 24 bp, Artificial Sequence
  1st STEP forward for MMGT1
cccactcccctttctaagaacact

SEQ ID NO: 374 - DNA, 23 bp, Artificial Sequence
  1st STEP reverse for MMGT1
tgaccttgccctgtccaataaat

SEQ ID NO: 375 - DNA, 24 bp, Artificial Sequence
  2nd STEP forward for MMGT1
tgcatacatcatctttcttgcccc

SEQ ID NO: 376 - DNA, 23 bp, Artificial Sequence
  2nd STEP reverse for MMGT1
agcatcttcctggttgtatgtgg

SEQ ID NO: 377 - DNA, 22 bp, Artificial Sequence
  1st STEP forward for SLC9A6
ttttgtgtgctaggggagggag

SEQ ID NO: 378 - DNA, 22 bp, Artificial Sequence
  1st STEP reverse for SLC9A6
aacttctgacgacaaagcctgc

SEQ ID NO: 379 - DNA, 22 bp, Artificial Sequence
  2nd STEP forward for SLC9A6
tggttgcactctgtagactgga

SEQ ID NO: 380 - DNA, 22 bp, Artificial Sequence
  2nd STEP reverse for SLC9A6
ctgactttggtgcagtgtggaa

SEQ ID NO: 381 - DNA, 18 bp, Artificial Sequence
  HK1338
gcgaacccgaggagatga

SEQ ID NO: 382 - DNA, 19 bp, Artificial Sequence
  HK1339
agatccaggcgctgtcctt

SEQ ID NO: 383 - DNA, 22 bp, Artificial Sequence
  HK1375
ccttcggatacagcaaattctt

SEQ ID NO: 384 - DNA, 22 bp, Artificial Sequence
  HK1376
gcagggaggagtgttttatacc

SEQ ID NO: 385 - DNA, 23 bp, Artificial Sequence
  HY2671
cactgtgttggcgtacaggtctt

SEQ ID NO: 386 - DNA, 22 bp, Artificial Sequence
  HY2672
ctgaggcactcttccagccttc

SEQ ID NO: 387 - DNA, 24 bp, Artificial Sequence
  HY2223
acattgcattagtctccctttcac

SEQ ID NO: 388 - DNA, 24 bp, Artificial Sequence
  HY2224
aattgagttgttttgttgcctgaa